European Patent Specification EP 4 211 663 B1, published February 18, 2026. Title: A Scoring Method for an Anti-B7H4 Antibody-Drug Conjugate Therapy. Applicant: MEDIMMUNE LIMITED. The sequence listing filed with the application follows.

SEQUENCE LISTING (13 sequences)

SEQ ID NO: 1 - protein, 282 aa, Homo sapiens
MASLGQILFWSIISIIIILAGAIALIIGFGISGRHSITVTTVASAGNIGEDGILSCTFEPDIKLSDIVIQWLKEGVLGLVHEFKEGKDELSEQDEMFRGRTAVFADQVIVGNASLRLKNVQLTDAGTYKCYIITSKGKGNANLEYKTGAFSMPEVNVDYNASSETLRCEAPRWFPQPTVVWASQVDQGANFSEVSNTSFELNSENVTMKVVSVLYNVTINNTYSCMIENDIAKATGDIKVTESEIKRRSHLQLLNSKASLCVSSFFAISWALLPLSPYLMLK

SEQ ID NO: 2 - DNA, 858 bp, Homo sapiens
gccaccatggcttccctggggcagatcctcttctggagcataattagcatcatcattattctggctggagcaattgcactcatcattggctttggtatttcagggagacactccatcacagtcactactgtcgcctcagctgggaacattggggaggatggaatcctgagctgcacttttgaacctgacatcaaactttctgatatcgtgatacaatggctgaaggaaggtgttttaggcttggtccatgagttcaaagaaggcaaagatgagctgtcggagcaggatgaaatgttcagaggccggacagcagtgtttgctgatcaagtgatagttggcaatgcctctttgcggctgaaaaacgtgcaactcacagatgctggcacctacaaatgttatatcatcacttctaaaggcaaggggaatgctaaccttgagtataaaactggagccttcagcatgccggaagtgaatgtggactataatgccagctcagagaccttgcggtgtgaggctccccgatggttcccccagcccacagtggtctgggcatcccaagttgaccagggagccaacttctcggaagtctccaataccagctttgagctgaactctgagaatgtgaccatgaaggttgtgtctgtgctctacaatgttacgatcaacaacacatactcctgtatgattgaaaatgacattgccaaagcaacaggggatatcaaagtgacagaatcggagatcaaaaggcggagtcacctacagctgctaaactcaaaggcttctctgtgtgtctcttctttctttgccatcagctgggcacttctgcctctcagcccttacctgatgctaaaataataa

SEQ ID NO: 3 - DNA, 846 bp, Homo sapiens
atggcttccctggggcagatcctcttctggagcataattagcatcatcattattctggctggagcaattgcactcatcattggctttggtatttcagggagacactccatcacagtcactactgtcgcctcagctgggaacattggggaggatggaatcctgagctgcacttttgaacctgacatcaaactttctgatatcgtgatacaatggctgaaggaaggtgttttaggcttggtccatgagttcaaagaaggcaaagatgagctgtcggagcaggatgaaatgttcagaggccggacagcagtgtttgctgatcaagtgatagttggcaatgcctctttgcggctgaaaaacgtgcaactcacagatgctggcacctacaaatgttatatcatcacttctaaaggcaaggggaatgctaaccttgagtataaaactggagccttcagcatgccggaagtgaatgtggactataatgccagctcagagaccttgcggtgtgaggctccccgatggttcccccagcccacagtggtctgggcatcccaagttgaccagggagccaacttctcggaagtctccaataccagctttgagctgaactctgagaatgtgaccatgaaggttgtgtctgtgctctacaatgttacgatcaacaacacatactcctgtatgattgaaaatgacattgccaaagcaacaggggatatcaaagtgacagaatcggagatcaaaaggcggagtcacctacagctgctaaactcaaaggcttctctgtgtgtctcttctttctttgccatcagctgggcacttctgcctctcagcccttacctgatgctaaaa

SEQ ID NO: 4 - protein, 5 aa, Artificial Sequence
  Sythetic Peptide
GYYWN

SEQ ID NO: 5 - protein, 16 aa, Artificial Sequence
  Sythetic Peptide
EINHSGSTSYNPSLKS

SEQ ID NO: 6 - protein, 9 aa, Artificial Sequence
  Sythetic Peptide
VLYNWNVDS

SEQ ID NO: 7 - protein, 11 aa, Artificial Sequence
  Sythetic Peptide
RASQDIRNDVG

SEQ ID NO: 8 - protein, 7 aa, Artificial Sequence
  Sythetic Peptide
AASRLQS

SEQ ID NO: 9 - protein, 9 aa, Artificial Sequence
  Sythetic Peptide
LQHNSYPRT

SEQ ID NO: 10 - protein, 117 aa, Artificial Sequence
  Sythetic Peptide
QVQLQQWGAGLLKPSETLSLACTVYGGSFSGYYWNWIRQPPGKGLEWIGEINHSGSTSYNPSLKSRVTISVDTSKNQFSLKLSSVTAADTAVYYCARVLYNWNVDSWGQGTLVTVSS

SEQ ID NO: 11 - protein, 107 aa, Artificial Sequence
  Sythetic Peptide
DIQMTQSPSSLSASVGDRVTITCRASQDIRNDVGWYQQKPGKAPKRLIYAASRLQSGVPSRFSGSGSGTEFTLTISSLQPEDFATYYCLQHNSYPRTFGQGTKVEIK

SEQ ID NO: 12 - protein, 447 aa, Artificial Sequence
  Sythetic Peptide
QVQLQQWGAGLLKPSETLSLACTVYGGSFSGYYWNWIRQPPGKGLEWIGEINHSGSTSYNPSLKSRVTISVDTSKNQFSLKLSSVTAADTAVYYCARVLYNWNVDSWGQGTLVTVSSASTKGPSVFPLAPSSKSTSGGTAALGCLVKDYFPEPVTVSWNSGALTSGVHTFPAVLQSSGLYSLSSVVTVPSSSLGTQTYICNVNHKPSNTKVDKRVEPKSCDKTHTCPPCPAPELLGGPSVFLFPPKPKDTLMISRTPEVTCVVVDVSHEDPEVKFNWYVDGVEVHNAKTKPREEQYNSTYRVVSVLTVLHQDWLNGKEYKCKVSNKALPAPIEKTISKAKGQPREPQVYTLPPSREEMTKNQVSLTCLVKGFYPSDIAVEWESNGQPENNYKTTPPVLDSDGSFFLYSKLTVDKSRWQQGNVFSCSVMHEALHNHYTQKSLSLSPGK

SEQ ID NO: 13 - protein, 214 aa, Artificial Sequence
  Sythetic Peptide
DIQMTQSPSSLSASVGDRVTITCRASQDIRNDVGWYQQKPGKAPKRLIYAASRLQSGVPSRFSGSGSGTEFTLTISSLQPEDFATYYCLQHNSYPRTFGQGTKVEIKRTVAAPSVFIFPPSDEQLKSGTASVVCLLNNFYPREAKVQWKVDNALQSGNSQESVTEQDSKDSTYSLSSTLTLSKADYEKHKVYACEVTHQGLSSPVTKSFNRGEC